European Patent Specification EP 3 313 862 B9, published October 4, 2023. Title: BROAD-SPECTRUM ANTI-INFECTIVE PEPTIDES. Applicant: Nanyang Technological University. Application TBA. The sequence listing filed with the application follows.

SEQUENCE LISTING (40 sequences)

SEQ ID NO: 1 - protein, 16 aa, Artificial Sequence
  Anti-infective peptides - TSG001
SGSWLRDVWTWLQSKL

SEQ ID NO: 2 - protein, 16 aa, Artificial Sequence
  Anti-infective peptides - TSG002
GSSWLRDVWTWLQSKL

SEQ ID NO: 3 - protein, 16 aa, Artificial Sequence
  Anti-infective peptides - TSG003
GSSWLRDVWTWLQSAL

SEQ ID NO: 4 - protein, 16 aa, Artificial Sequence
  Anti-infective peptides - TSG004
GSSWLRDVWTKLQSWL

SEQ ID NO: 5 - protein, 16 aa, Artificial Sequence
  Anti-infective peptides - TSG005
GSSWLRDIWTKLQSWL

SEQ ID NO: 6 - protein, 16 aa, Artificial Sequence
  Anti-infective peptides - TSG006
GSSWLRDIWTALQSWL

SEQ ID NO: 7 - protein, 16 aa, Artificial Sequence
  Anti-infective peptide - TSG007
GSSWLRDILTALQSLL

SEQ ID NO: 8 - protein, 16 aa, Artificial Sequence
  Anti-infective peptide - TSG008
AGSWLRDIWTWLQSAL

SEQ ID NO: 9 - protein, 16 aa, Artificial Sequence
  Anti-infective peptide - TSG009
AGSWLRDILTLLQSAL

SEQ ID NO: 10 - protein, 27 aa, Artificial Sequence
  AH peptide
SGSWLRDVWDWICTVLTDFKTWLQSKL

SEQ ID NO: 11 - protein, 18 aa, Artificial Sequence
  C5A peptide
SWLRDIWDWICEVLSDFK

SEQ ID NO: 12 - protein, 16 aa, Artificial Sequence
  Anti-infective peptides consensus sequence
  misc_feature (1)..(2): Xaa = Ser, Gly or Ala
  misc_feature (1)..(2): Xaa = Ser or Gly
  misc_feature (8)..(8): Xaa = Val or Ile
  misc_feature (9)..(9): Xaa = Trp or Leu
  misc_feature (11)..(11): Xaa = Trp, Lys, Ala or Leu
  misc_feature (15)..(15): Xaa = Trp, Lys, Leu or Ala
XXSWLRDXXTXLQSXL

SEQ ID NO: 13 - protein, 16 aa, Artificial Sequence
  Anti-infective peptide consensus sequence
  misc_feature (1)..(2): Xaa = Ser or Gly
  misc_feature (8)..(8): Xaa = Val
  misc_feature (9)..(9): Xaa = Trp
  misc_feature (11)..(11): Xaa = Trp or Lys
  misc_feature (15)..(15): Xaa = Trp, Lys or Ala
XXSWLRDXXTXLQSXL

SEQ ID NO: 14 - protein, 16 aa, Artificial Sequence
  Anti-infective peptide consensus sequence
  misc_feature (1)..(2): Xaa = Ser or Gly
  misc_feature (8)..(8): Xaa = Val
  misc_feature (9)..(9): Xaa = Trp
  misc_feature (11)..(11): Xaa = Trp
  misc_feature (15)..(15): Xaa = Lys or Ala
XXSWLRDXXTXLQSXL

SEQ ID NO: 15 - protein, 16 aa, Artificial Sequence
  Anti-infective peptide consensus sequence
  misc_feature (1)..(2): Xaa = Ser or Gly
  misc_feature (8)..(8): Xaa = Val or Ile
  misc_feature (9)..(9): Xaa = Trp
  misc_feature (11)..(11): Xaa = Trp or Ala
  misc_feature (15)..(15): Xaa = Trp or Lys
XXSWLRDXXTXLQSXL

SEQ ID NO: 16 - protein, 16 aa, Artificial Sequence
  Anti-infective peptide consensus sequence
  misc_feature (1)..(2): Xaa = Ser or Gly
  misc_feature (8)..(8): Xaa = Val or Ile
  misc_feature (9)..(9): Xaa = Trp
  misc_feature (11)..(11): Xaa = Trp, Lys or Ala
  misc_feature (15)..(15): Xaa = Trp, Lys or Ala
XXSWLRDXXTXLQSXL

SEQ ID NO: 17 - protein, 16 aa, Artificial Sequence
  Anti-infective peptide consensus sequence
  misc_feature (1)..(2): Xaa = Ser or Gly
  misc_feature (8)..(8): Xaa = Val or Ile
  misc_feature (9)..(9): Xaa = Trp
  misc_feature (11)..(11): Xaa = Trp or Ala
  misc_feature (15)..(15): Xaa = Trp, Lys or Ala
XXSWLRDXXTXLQSXL

SEQ ID NO: 18 - protein, 16 aa, Artificial Sequence
  Anti-infective peptide consensus sequence
  misc_feature (1)..(2): Xaa = Gly, Pro or Ala
  misc_feature (8)..(8): Xaa = Val, Ile, Leu or Met
  misc_feature (9)..(9): Xaa = Trp, Phe, Tyr or His
  misc_feature (11)..(11): Xaa = Ala, Ser, Gly or Thr
  misc_feature (15)..(15): Xaa = Trp, Tyr or Phe
XXSWLRDXXTXLQSXL

SEQ ID NO: 19 - protein, 16 aa, Artificial Sequence
  Anti-infective peptide consensus sequence
  misc_feature (1)..(2): Xaa = Ser or Gly
  misc_feature (8)..(8): Xaa = Val or Ile
  misc_feature (9)..(9): Xaa = Trp
  misc_feature (11)..(11): Xaa = Trp, Lys or Ala
  misc_feature (15)..(15): Xaa = Trp or Lys
XXSWLRDXXTXLQSXL

SEQ ID NO: 20 - protein, 7 aa, Artificial Sequence
  C-teminal of C5A peptide
TWLQSKL

SEQ ID NO: 21 - protein, 16 aa, Artificial Sequence
  Anti-infective peptide consensus sequence
  misc_feature (1)..(2): Xaa is small amino acid
  misc_feature (8)..(8): Xaa is hydrophobic amino acid with an aliphatic side chain
  misc_feature (9)..(9): Xaa is hydrophobic amino acid
  misc_feature (11)..(11): Xaa is hydrophilic amino acid or polar amino acid
  misc_feature (15)..(15): Xaa is hydrophilic amino acid or polar amino acid
XXSWLRDXXTXLQSXL

SEQ ID NO: 22 - protein, 16 aa, Artificial Sequence
  Anti-infective peptide consensus sequence
  misc_feature (1)..(2): Xaa is small amino acid
  misc_feature (8)..(8): Xaa is hydrophobic amino acid with an aliphatic side chain
  misc_feature (9)..(9): Xaa is hydrophobic amino acid
  misc_feature (11)..(11): Xaa is hydrophilic amino acid
  misc_feature (15)..(15): Xaa is hydrophilic amino acid
XXSWLRDXXTXLQSXL

SEQ ID NO: 23 - protein, 16 aa, Artificial Sequence
  Anti-infective peptide consensus sequence
  misc_feature (1)..(2): Xaa is small amino acid
  misc_feature (8)..(8): Xaa is hydrophobic amino acid with an aliphatic side chain
  misc_feature (9)..(9): Xaa is hydrophobic amino acid
  misc_feature (11)..(11): Xaa is polar amino acid
  misc_feature (15)..(15): Xaa is polar amino acid
XXSWLRDXXTXLQSXL

SEQ ID NO: 24 - protein, 16 aa, Artificial Sequence
  Anti-infective peptide consensus sequence
  misc_feature (1)..(2): Xaa is small amino acid
  misc_feature (8)..(8): Xaa is hydrophobic amino acid with an aliphatic side chain
  misc_feature (9)..(9): Xaa is hydrophobic amino acid
  misc_feature (11)..(11): Xaa is hydrophilic amino acid
  misc_feature (15)..(15): Xaa is polar amino acid
XXSWLRDXXTXLQSXL

SEQ ID NO: 25 - protein, 16 aa, Artificial Sequence
  Anti-infective peptide consensus sequence
  misc_feature (1)..(2): Xaa is small amino acid
  misc_feature (8)..(8): Xaa is hydrophobic amino acid with an aliphatic side chain
  misc_feature (9)..(9): Xaa is hydrophobic amino acid
  misc_feature (11)..(11): Xaa is polar amino acid
  misc_feature (15)..(15): Xaa is hydrophilic amino acid
XXSWLRDXXTXLQSXL

SEQ ID NO: 26 - protein, 16 aa, Artificial Sequence
  Anti-infective peptide consensus sequence
  misc_feature (1)..(2): Xaa is conservative amino acid substitution for serine, glycine or alanine
  misc_feature (8)..(8): Xaa is conservative amino acid substitution for valine or isoleucine
  misc_feature (9)..(9): Xaa is conservative amino acid substitution for tryptophan or leucine
  misc_feature (11)..(11): Xaa is conservative amino acid substitution for tryptophan, lysine, alanine or leucine
  misc_feature (15)..(15): Xaa is conservative amino acid substitution for tryptophan, lysine, alanine or leucine
XXSWLRDXXTXLQSXL

SEQ ID NO: 27 - protein, 16 aa, Artificial Sequence
  Anti-infective peptide consensus sequence
  misc_feature (1)..(2): Xaa = Ala, Cys, Gly, Pro, Ser or Thr
  misc_feature (8)..(8): Xaa = Ala, Ile, Leu, Pro or Val
  misc_feature (9)..(9): Xaa = Trp, Phe, Tyr, His, Ala, Ile, Leu, Pro or Val
  misc_feature (11)..(11): Xaa = Trp, Phe, Tyr or His
  misc_feature (15)..(15): Xaa = Trp, Phe, Tyr or His
XXSWLRDXXTXLQSXL

SEQ ID NO: 28 - protein, 16 aa, Artificial Sequence
  Anti-infective peptide consensus sequence
  misc_feature (1)..(2): Xaa = Ala, Cys, Gly, Pro, Ser or Thr
  misc_feature (8)..(8): Xaa = Ala, Ile, Leu, Pro or Val
  misc_feature (9)..(9): Xaa = Trp, Phe, Tyr, His, Ala, Ile, Leu, Pro or Val
  misc_feature (11)..(11): Xaa = Trp, Phe, Tyr or His
  misc_feature (15)..(15): Xaa = Lys, Tyr, Arg, His, Asn, Gln, Ser or Thr
XXSWLRDXXTXLQSXL

SEQ ID NO: 29 - protein, 16 aa, Artificial Sequence
  Anti-infective peptide consensus sequence
  misc_feature (1)..(2): Xaa = Ala, Cys, Gly, Pro, Ser or Thr
  misc_feature (8)..(8): Xaa = Ala, Ile, Leu, Pro or Val
  misc_feature (9)..(9): Xaa = Trp, Phe, Tyr, His, Ala, Ile, Leu, Pro or Val
  misc_feature (11)..(11): Xaa = Trp, Phe, Tyr or His
  misc_feature (15)..(15): Xaa = Ala, Cys, Gly, Pro, Ser, Ile, Leu, Val or Thr
XXSWLRDXXTXLQSXL

SEQ ID NO: 30 - protein, 16 aa, Artificial Sequence
  Anti-infective peptide consensus sequence
  misc_feature (1)..(2): Xaa = Ala, Cys, Gly, Pro, Ser or Thr
  misc_feature (8)..(8): Xaa = Ala, Ile, Leu, Pro or Val
  misc_feature (9)..(9): Xaa = Trp, Phe, Tyr, His, Ala, Ile, Leu, Pro or Val
  misc_feature (11)..(11): Xaa = Lys, Tyr, Arg, His, Asn, Gln, Ser or Thr
  misc_feature (15)..(15): Xaa = Trp, Phe, Tyr or His
XXSWLRDXXTXLQSXL

SEQ ID NO: 31 - protein, 16 aa, Artificial Sequence
  Anti-infective peptide consensus sequence
  misc_feature (1)..(2): Xaa = Ala, Cys, Gly, Pro, Ser or Thr
  misc_feature (8)..(8): Xaa = Ala, Ile, Leu, Pro or Val
  misc_feature (9)..(9): Xaa = Trp, Phe, Tyr, His, Ala, Ile, Leu, Pro or Val
  misc_feature (11)..(11): Xaa = Lys, Tyr, Arg, His, Asn, Gln, Ser or Thr
  misc_feature (15)..(15): Xaa = Lys, Tyr, Arg, His, Asn, Gln, Ser or Thr
XXSWLRDXXTXLQSXL

SEQ ID NO: 32 - protein, 16 aa, Artificial Sequence
  Anti-infective peptide consensus sequence
  misc_feature (1)..(2): Xaa = Ala, Cys, Gly, Pro, Ser or Thr
  misc_feature (8)..(8): Xaa = Ala, Ile, Leu, Pro or Val
  misc_feature (9)..(9): Xaa = Trp, Phe, Tyr, His, Ala, Ile, Leu, Pro or Val
  misc_feature (11)..(11): Xaa = Lys, Tyr, Arg, His, Asn, Gln, Ser or Thr
  misc_feature (15)..(15): Xaa = Ala, Cys, Gly, Pro, Ser, Ile, Leu, Val or Thr
XXSWLRDXXTXLQSXL

SEQ ID NO: 33 - protein, 16 aa, Artificial Sequence
  Anti-infective peptide consensus sequence
  misc_feature (1)..(2): Xaa = Ala, Cys, Gly, Pro, Ser or Thr
  misc_feature (8)..(8): Xaa = Ala, Ile, Leu, Pro or Val
  misc_feature (9)..(9): Xaa = Trp, Phe, Tyr, His, Ala, Ile, Leu, Pro or Val
  misc_feature (11)..(11): Xaa = Ala, Cys, Gly, Pro, Ser, Ile, Leu, Val or Thr
  misc_feature (15)..(15): Xaa = Trp, Phe, Tyr or His
XXSWLRDXXTXLQSXL

SEQ ID NO: 34 - protein, 16 aa, Artificial Sequence
  Anti-infective peptide consensus sequence
  misc_feature (1)..(2): Xaa = Ala, Cys, Gly, Pro, Ser or Thr
  misc_feature (8)..(8): Xaa = Ala, Ile, Leu, Pro or Val
  misc_feature (9)..(9): Xaa = Trp, Phe, Tyr, His, Ala, Ile, Leu, Pro or Val
  misc_feature (11)..(11): Xaa = Ala, Cys, Gly, Pro, Ser, Ile, Leu, Val or Thr
  misc_feature (15)..(15): Xaa = Lys, Tyr, Trp, Arg, His, Asn, Gln, Ser or Thr
XXSWLRDXXTXLQSXL

SEQ ID NO: 35 - protein, 16 aa, Artificial Sequence
  Anti-infective peptide consensus sequence
  misc_feature (1)..(2): Xaa = Ala, Cys, Gly, Pro, Ser or Thr
  misc_feature (8)..(8): Xaa = Ala, Ile, Leu, Pro or Val
  misc_feature (9)..(9): Xaa = Trp, Phe, Tyr, His, Ala, Ile, Leu, Pro or Val
  misc_feature (11)..(11): Xaa = Ala, Cys, Gly, Pro, Ser, Ile, Leu, Val or Thr
  misc_feature (15)..(15): Xaa = Ala, Cys, Gly, Pro, Ser, Ile, Leu, Val or Thr
XXSWLRDXXTXLQSXL

SEQ ID NO: 36 - protein, 16 aa, Artificial Sequence
  Anti-infective peptide consensus sequence
  misc_feature (1)..(2): Xaa = Gly, Pro or Ala
  misc_feature (8)..(8): Xaa = Val, Ile, Leu or Met
  misc_feature (9)..(9): Xaa = Trp, Phe, Tyr or His
  misc_feature (11)..(11): Xaa = Trp, Tyr or Phe
  misc_feature (15)..(15): Xaa = Lys, Arg, Gln, Glu or Asn
XXSWLRDXXTXLQSXL

SEQ ID NO: 37 - protein, 16 aa, Artificial Sequence
  Anti-infective peptide consensus sequence
  misc_feature (1)..(1): Xaa = Ser, Thr, Ala or Gln
  misc_feature (2)..(2): Xaa = Gly, Pro or Ala
  misc_feature (8)..(8): Xaa = Val, Ile, Leu or Met
  misc_feature (9)..(9): Xaa = Trp, Phe, Tyr or His
  misc_feature (11)..(11): Xaa = Trp, Tyr or Phe
  misc_feature (15)..(15): Xaa = Lys, Arg, Gln, Glu or Asn
XXSWLRDXXTXLQSXL

SEQ ID NO: 38 - protein, 16 aa, Artificial Sequence
  Anti-infective peptide consensus sequence
  misc_feature (1)..(2): Xaa = Gly, Pro or Ala
  misc_feature (8)..(8): Xaa = Val, Ile, Leu or Met
  misc_feature (9)..(9): Xaa = Trp, Phe, Tyr or His
  misc_feature (11)..(11): Xaa = Lys, Arg, Gln, Glu or Asn
  misc_feature (15)..(15): Xaa = Trp, Tyr or Phe
XXSWLRDXXTXLQSXL

SEQ ID NO: 39 - protein, 16 aa, Artificial Sequence
  Anti-infective peptide consensus sequence
  misc_feature (1)..(1): Xaa = Ser, Thr, Ala or Gln
  misc_feature (2)..(2): Xaa = Gly, Pro or Ala
  misc_feature (8)..(8): Xaa = Val, Ile, Leu or Met
  misc_feature (9)..(9): Xaa = Trp, Phe, Tyr or His
  misc_feature (11)..(11): Xaa = Lys, Arg, Gln, Glu or Asn
  misc_feature (15)..(15): Xaa = Trp, Tyr or Phe
XXSWLRDXXTXLQSXL

SEQ ID NO: 40 - protein, 16 aa, Artificial Sequence
  Anti-infective peptide consensus sequence
  misc_feature (1)..(1): Xaa = Ser, Thr, Ala or Gln
  misc_feature (2)..(2): Xaa = Gly, Pro or Ala
  misc_feature (8)..(8): Xaa = Val, Ile, Leu or Met
  misc_feature (9)..(9): Xaa = Trp, Phe, Tyr or His
  misc_feature (11)..(11): Xaa = Ala, Ser, Gly or Thr
  misc_feature (15)..(15): Xaa = Trp, Tyr or Phe
XXSWLRDXXTXLQSXL